European Patent Application EP 4 410 981 A1, published August 7, 2024. Title: Enzyme agent for collagen tripeptide production or cartilage degradation. Applicant: AMANO ENZYME INC. The sequence listing filed with the application follows.

SEQUENCE LISTING (10 sequences)

SEQ ID NO: 1 - protein, 1042 aa, Lysinibacillus fusiformis
AEKTPYNVLQMKPIGIEMSKDEMVHSTMAEETLSYEERLEMGDFSQRPAPIMEQMDTQQLQEQYSMAELNNMSNRELIHTLGSIRWYQITDLFQFNDDTKAFYQNEERMQVIINELGNRGSSFTKDDSKGIETFVEVLRSAFYVAFYNNELGYLNERSFQDKCLPALNEIAKNPNFKLGTDEQDKVVSAYGKLIGNASSDVETVQHATNILKQYNENLSTYESENSKGQAIYDIIHGIDYDLQSYLYDTRKEANTTMWYGKIDSFIEEVNNIALIHNVTDSNSWLINNGIYYAGRLGQFHSNPNKGLEVVSQAMHMYPYLSEAYFVAVEQITTNYGGRDLNGNTVDLQKVREEGKKQYLPKTYTFDDGSIVFKTGDQVTEDKIQRLYWAAKEVKAQYHRVIGNDQALEPGNADDILTVVIYNSPDQYRLNRQLYGYETNNGGIYIEETGTFFTYERTPEQSIYSLEELFRHEYTHFLQGRFEVPGLFGTGDMYQNERLTWFQEGNAEFFAGSTRTNDVVPRKSIISGLSHDPSQRYTAEQTMFATYGSWDFYNYSFALQSYMYTHQFDMFDRIQDLIRANDVKNYDAYRDTLSKDSQLNMEYQAYMQQLIDNQETYEVPQVAEDYLMPHEPKALNEVQQEIVDIAHVKDANMTKHQSQFFNTFTLEGTYVGSATQGESQDWKTMSKQVNQMLEQLSQKEWSGYKTMTAYFVNYRVNAANQFEYDVVFHGVSTDDGETQAPIVQVNGPYTGMINEKIQFNSDGSKDTDGEIVSYLWDFGDGATSEAANPTHVYENEGTYKVTLTVKNNKGQESKGQTTATVQKGGQTGQEHAMTIPFNKPIKGSLIENDTNVYQFDITSLEEIDISVVNENQIGMTWVLYHESDKENYVAYGQEDGQTIKGKYNAKPGKYYLYVYKFDDENGTYTVQVQNSTKTEIEPNNRPEEATMLPFHTPLSGSLMEDDHTDVYEFNVTSPKEIDISVLNENQIGMTWVLYHESDSQNYASFGQEDGNMINGKLNAKPGKYYLYVYKFENENGTYTVHVQ

SEQ ID NO: 2 - protein, 1072 aa, Lysinibacillus fusiformis
MKKKFTFNQLLIGVSTMAISLGGLQAEASAAEKTPYNVLQMKPIGIEMSKDEMVHSTMAEETLSYEERLEMGDFSQRPAPIMEQMDTQQLQEQYSMAELNNMSNRELIHTLGSIRWYQITDLFQFNDDTKAFYQNEERMQVIINELGNRGSSFTKDDSKGIETFVEVLRSAFYVAFYNNELGYLNERSFQDKCLPALNEIAKNPNFKLGTDEQDKVVSAYGKLIGNASSDVETVQHATNILKQYNENLSTYESENSKGQAIYDIIHGIDYDLQSYLYDTRKEANTTMWYGKIDSFIEEVNNIALIHNVTDSNSWLINNGIYYAGRLGQFHSNPNKGLEVVSQAMHMYPYLSEAYFVAVEQITTNYGGRDLNGNTVDLQKVREEGKKQYLPKTYTFDDGSIVFKTGDQVTEDKIQRLYWAAKEVKAQYHRVIGNDQALEPGNADDILTVVIYNSPDQYRLNRQLYGYETNNGGIYIEETGTFFTYERTPEQSIYSLEELFRHEYTHFLQGRFEVPGLFGTGDMYQNERLTWFQEGNAEFFAGSTRTNDVVPRKSIISGLSHDPSQRYTAEQTMFATYGSWDFYNYSFALQSYMYTHQFDMFDRIQDLIRANDVKNYDAYRDTLSKDSQLNMEYQAYMQQLIDNQETYEVPQVAEDYLMPHEPKALNEVQQEIVDIAHVKDANMTKHQSQFFNTFTLEGTYVGSATQGESQDWKTMSKQVNQMLEQLSQKEWSGYKTMTAYFVNYRVNAANQFEYDVVFHGVSTDDGETQAPIVQVNGPYTGMINEKIQFNSDGSKDTDGEIVSYLWDFGDGATSEAANPTHVYENEGTYKVTLTVKNNKGQESKGQTTATVQKGGQTGQEHAMTIPFNKPIKGSLIENDTNVYQFDITSLEEIDISVVNENQIGMTWVLYHESDKENYVAYGQEDGQTIKGKYNAKPGKYYLYVYKFDDENGTYTVQVQNSTKTEIEPNNRPEEATMLPFHTPLSGSLMEDDHTDVYEFNVTSPKEIDISVLNENQIGMTWVLYHESDSQNYASFGQEDGNMINGKLNAKPGKYYLYVYKFENENGTYTVHVQ

SEQ ID NO: 3 - DNA, 3129 bp, Lysinibacillus fusiformis
  source 1..3129: mol_type = genomic DNA
gcagaaaaaacgccgtataatgtattacaaatgaaacccattggcatagaaatgtcgaaagatgaaatggtgcattcgacaatggctgaagaaacattatcctatgaagaacgtttagaaatgggagatttttcacaacgtccagcaccaattatggaacagatggatacacagcaattgcaggagcagtactcgatggcagagcttaataatatgagcaatcgtgagctcatccatacgcttggcagtatccgttggtaccaaattacagacttattccaattcaatgatgacacaaaagctttttatcaaaatgaagagcgcatgcaagtaatcatcaatgaattaggtaatagaggaagttcgtttacgaaggatgattcaaaggggatcgaaacatttgttgaggtactgcgttctgctttttatgtagcgttttataataatgaactaggttatttaaatgagagaagtttccaagataagtgtttaccagcattaaatgaaatagccaaaaatccaaactttaaacttggtacagatgagcaagataaagttgtatctgcctatggaaaattaataggtaatgcttctagtgatgtggaaaccgttcaacatgctacgaacattttaaaacaatataatgaaaatctttctacctatgaaagtgagaattcaaaaggacaagctatttacgatataatacacggcattgattatgatttgcagtcttatttatatgacactcgtaaagaggccaatacaacgatgtggtatgggaagattgatagcttcatagaggaagttaataacattgccctaatacataatgtgacggatagcaatagttggttaattaataatggcatttattatgcagggcgtttagggcagttccatagcaatccgaataagggtttagaagtcgtttcacaagcgatgcatatgtatccctatttaagtgaagcttattttgtggcagtagagcaaattacgacaaattatggtggacgtgacttaaacggaaatacggttgatttacaaaaagtacgtgaagaaggaaaaaaacagtatctaccgaaaacatatacatttgatgatggatcaattgtattcaaaacgggagatcaagtaacggaagataaaattcaaagattatactgggctgcaaaagaggtaaaggcacaatatcatcgtgtaatcgggaatgatcaagcactagagcctggtaatgctgacgatatcttaaccgttgtcatttataactctcccgatcagtaccgattaaaccgacaattgtacggatatgaaacaaataatggtggtatttatattgaagagactggaacattctttacatatgaacgtacacctgagcaaagtatttatagcttagaagagctgttccgtcatgaatatacgcactttttacaaggtagatttgaggtgcctggtctattcgggacgggtgatatgtatcaaaatgagcgactaacatggttccaggaagggaatgcagaattttttgcagggtcaacacgtacaaatgacgttgtgcctcgtaagagcattattagtggattgtcacatgatccatcacaacgctatacagctgaacaaacaatgtttgcgacatatggttcctgggatttttacaattattcatttgctttacagtcttatatgtatactcatcaattcgatatgtttgatagaattcaagatttaattcgcgcgaacgatgtgaaaaattatgatgcctatcgtgacactttaagtaaagattcacagctgaatatggaatatcaagcgtatatgcagcaattgatcgataaccaagaaacatacgaagtaccacaagtagcagaggattatttaatgccgcatgaaccaaaagcgttaaacgaagtacagcaagaaattgtcgatattgcacatgtgaaagatgcaaatatgacgaaacaccagtctcaattttttaatacgtttacactcgagggaacatatgtaggtagtgcaacacagggtgaatctcaagattggaaaacgatgagtaagcaagtaaaccaaatgctggagcaactgtctcaaaaagagtggagcggctataaaacaatgactgcgtactttgtcaactatcgtgtaaatgcggcaaaccagttcgagtatgatgtagtcttccacggtgtttccactgatgacggagaaacgcaagcaccaattgtacaggtaaatggtccatatactggcatgatcaatgaaaaaattcaatttaacagtgatgggtcaaaggatacggatggagaaatagtttcttatctttgggattttggtgatggtgcaacaagtgaagcagcaaatcctactcatgtatacgaaaatgaaggaacttacaaagtgacgttaaccgtgaaaaataataagggacaagaaagtaaagggcaaacaactgccactgtacagaaaggaggacaaacagggcaagaacatgcgatgaccattccatttaataaaccaataaaaggtagtttgatagaaaacgatacaaatgtctatcaatttgacattacatcgctagaagaaatagatatttctgtcgtaaatgaaaatcaaattggcatgacatgggtgctttatcatgaatctgataaggaaaactatgtagcgtatggacaggaagatggacagacaataaaaggtaagtacaatgcgaaaccaggaaagtactatttatacgtttataagtttgatgatgaaaatggaacatataccgttcaagtacaaaatagtacaaaaacggagatagaaccaaacaatcgtccagaagaagccactatgcttccatttcatacaccactaagcggtagtttaatggaggatgatcatacggatgtatacgaattcaatgttacatctcctaaagaaatagatatatctgttttaaatgaaaaccaaattggcatgacatgggtgctttatcatgaatcagatagccaaaattatgcgtcttttggacaggaagacggaaacatgataaacggtaaattgaatgcaaagcctggaaagtattatttatatgtttataaatttgaaaatgagaacggaacatataccgttcatgtacagtaa

SEQ ID NO: 4 - DNA, 3219 bp, Lysinibacillus fusiformis
  source 1..3219: mol_type = genomic DNA
atgaagaaaaaatttacattcaatcagttgttaattggggttagtacaatggccatttcgttaggtggattacaggcggaagcatcggcagcagaaaaaacgccgtataatgtattacaaatgaaacccattggcatagaaatgtcgaaagatgaaatggtgcattcgacaatggctgaagaaacattatcctatgaagaacgtttagaaatgggagatttttcacaacgtccagcaccaattatggaacagatggatacacagcaattgcaggagcagtactcgatggcagagcttaataatatgagcaatcgtgagctcatccatacgcttggcagtatccgttggtaccaaattacagacttattccaattcaatgatgacacaaaagctttttatcaaaatgaagagcgcatgcaagtaatcatcaatgaattaggtaatagaggaagttcgtttacgaaggatgattcaaaggggatcgaaacatttgttgaggtactgcgttctgctttttatgtagcgttttataataatgaactaggttatttaaatgagagaagtttccaagataagtgtttaccagcattaaatgaaatagccaaaaatccaaactttaaacttggtacagatgagcaagataaagttgtatctgcctatggaaaattaataggtaatgcttctagtgatgtggaaaccgttcaacatgctacgaacattttaaaacaatataatgaaaatctttctacctatgaaagtgagaattcaaaaggacaagctatttacgatataatacacggcattgattatgatttgcagtcttatttatatgacactcgtaaagaggccaatacaacgatgtggtatgggaagattgatagcttcatagaggaagttaataacattgccctaatacataatgtgacggatagcaatagttggttaattaataatggcatttattatgcagggcgtttagggcagttccatagcaatccgaataagggtttagaagtcgtttcacaagcgatgcatatgtatccctatttaagtgaagcttattttgtggcagtagagcaaattacgacaaattatggtggacgtgacttaaacggaaatacggttgatttacaaaaagtacgtgaagaaggaaaaaaacagtatctaccgaaaacatatacatttgatgatggatcaattgtattcaaaacgggagatcaagtaacggaagataaaattcaaagattatactgggctgcaaaagaggtaaaggcacaatatcatcgtgtaatcgggaatgatcaagcactagagcctggtaatgctgacgatatcttaaccgttgtcatttataactctcccgatcagtaccgattaaaccgacaattgtacggatatgaaacaaataatggtggtatttatattgaagagactggaacattctttacatatgaacgtacacctgagcaaagtatttatagcttagaagagctgttccgtcatgaatatacgcactttttacaaggtagatttgaggtgcctggtctattcgggacgggtgatatgtatcaaaatgagcgactaacatggttccaggaagggaatgcagaattttttgcagggtcaacacgtacaaatgacgttgtgcctcgtaagagcattattagtggattgtcacatgatccatcacaacgctatacagctgaacaaacaatgtttgcgacatatggttcctgggatttttacaattattcatttgctttacagtcttatatgtatactcatcaattcgatatgtttgatagaattcaagatttaattcgcgcgaacgatgtgaaaaattatgatgcctatcgtgacactttaagtaaagattcacagctgaatatggaatatcaagcgtatatgcagcaattgatcgataaccaagaaacatacgaagtaccacaagtagcagaggattatttaatgccgcatgaaccaaaagcgttaaacgaagtacagcaagaaattgtcgatattgcacatgtgaaagatgcaaatatgacgaaacaccagtctcaattttttaatacgtttacactcgagggaacatatgtaggtagtgcaacacagggtgaatctcaagattggaaaacgatgagtaagcaagtaaaccaaatgctggagcaactgtctcaaaaagagtggagcggctataaaacaatgactgcgtactttgtcaactatcgtgtaaatgcggcaaaccagttcgagtatgatgtagtcttccacggtgtttccactgatgacggagaaacgcaagcaccaattgtacaggtaaatggtccatatactggcatgatcaatgaaaaaattcaatttaacagtgatgggtcaaaggatacggatggagaaatagtttcttatctttgggattttggtgatggtgcaacaagtgaagcagcaaatcctactcatgtatacgaaaatgaaggaacttacaaagtgacgttaaccgtgaaaaataataagggacaagaaagtaaagggcaaacaactgccactgtacagaaaggaggacaaacagggcaagaacatgcgatgaccattccatttaataaaccaataaaaggtagtttgatagaaaacgatacaaatgtctatcaatttgacattacatcgctagaagaaatagatatttctgtcgtaaatgaaaatcaaattggcatgacatgggtgctttatcatgaatctgataaggaaaactatgtagcgtatggacaggaagatggacagacaataaaaggtaagtacaatgcgaaaccaggaaagtactatttatacgtttataagtttgatgatgaaaatggaacatataccgttcaagtacaaaatagtacaaaaacggagatagaaccaaacaatcgtccagaagaagccactatgcttccatttcatacaccactaagcggtagtttaatggaggatgatcatacggatgtatacgaattcaatgttacatctcctaaagaaatagatatatctgttttaaatgaaaaccaaattggcatgacatgggtgctttatcatgaatcagatagccaaaattatgcgtcttttggacaggaagacggaaacatgataaacggtaaattgaatgcaaagcctggaaagtattatttatatgtttataaatttgaaaatgagaacggaacatataccgttcatgtacagtaa

SEQ ID NO: 5 - protein, 987 aa, Lysinibacillus fusiformis
DTQQLQEQYSMAELNNMSNRELIHTLGSIRWYQITDLFQFNDDTKAFYQNEERMQVIINELGNRGNSFTKEDSKGIETFVEVLRSAFYVAFYNNELGYLNERSFQDKCLPALNEIAKNPNFKLGTDEQDKVVSAYGKLIGNASSDVETVQHATNILKQYNENLSTYESENSKGQAIYDIIHGIDYDLQSYLYDTRKEANTTMWYGKIDSFIEEVNNIALIHNVTDSNSWLINNGIYYAGRLGQFHSNPNKGLEVVTQAMHMYPYLSEAYFVAVEQITTNYGGRDLNGNTVDLQKVREEGKKQYLPKTYTFDDGSIVFKTGDQVTEDKIQRLYWAAKEVKAQYHRVIGNDQALEPGNADDILTVVIYNSPDQYRLNRQLYGYETNNGGIYIEETGTFFTYERTPEQSIYSLEELFRHEYTHFLQGRFEVPGLFGTGDMYQNERLTWFQEGNAEFFAGSTRTNDVVPRKSIISGLSQDPSQRYTAEQTMFATYGSWDFYNYSFALQSYMYTHQFDMFDRIQDLIRANDVKNYDAYRDTLSKDSQLNMEYQAYMQQLIDNQETYEVPQVAEDYLMPHEPKALNEVQQEIVDIAHVKDANMTKHQSQFFNTFTLEGTYVGSATQGESQDWKTMSKQVNQMLEQLSQKEWSGYKTMTAYFVNYRVNAANQFEYDVVFHGVSTDDGETQAPIVQVNGPYTGMINEKIQFNSDGSKDTDGEIVSYLWDFGDGATSEAANPTHVYENEGTYKVTLTVKNNKGQESKGQTTATVQKGGQTGQEHAMIIPFNKPLKGSLIENDTNVYQFDITSPEEIDISVVNENQIGMTWVLYHESDKENYVAYGQEDGQTIKGKYNAKPGKYYLYVYKFDDEDGTYTVQVQNSTKTEIEPNNRPEEATMLPFHTPLSGSLMEDDHTDVYEFNVTSPKEIDISVLNENQIGMTWVLYHESDSQNYASFGQEDGNMINGKLNAKPGKYYLYVYKFENENGTYTVHVQ

SEQ ID NO: 6 - protein, 1072 aa, Lysinibacillus fusiformis
MKKKFTFNQLLIGVSTMAISLGGLQAEASAAEKTPYNVLQMKPIGIEMSKDEMVHSTMAEETLSYEERLEMGDFSQRPAPIMEQMDTQQLQEQYSMAELNNMSNRELIHTLGSIRWYQITDLFQFNDDTKAFYQNEERMQVIINELGNRGNSFTKEDSKGIETFVEVLRSAFYVAFYNNELGYLNERSFQDKCLPALNEIAKNPNFKLGTDEQDKVVSAYGKLIGNASSDVETVQHATNILKQYNENLSTYESENSKGQAIYDIIHGIDYDLQSYLYDTRKEANTTMWYGKIDSFIEEVNNIALIHNVTDSNSWLINNGIYYAGRLGQFHSNPNKGLEVVTQAMHMYPYLSEAYFVAVEQITTNYGGRDLNGNTVDLQKVREEGKKQYLPKTYTFDDGSIVFKTGDQVTEDKIQRLYWAAKEVKAQYHRVIGNDQALEPGNADDILTVVIYNSPDQYRLNRQLYGYETNNGGIYIEETGTFFTYERTPEQSIYSLEELFRHEYTHFLQGRFEVPGLFGTGDMYQNERLTWFQEGNAEFFAGSTRTNDVVPRKSIISGLSQDPSQRYTAEQTMFATYGSWDFYNYSFALQSYMYTHQFDMFDRIQDLIRANDVKNYDAYRDTLSKDSQLNMEYQAYMQQLIDNQETYEVPQVAEDYLMPHEPKALNEVQQEIVDIAHVKDANMTKHQSQFFNTFTLEGTYVGSATQGESQDWKTMSKQVNQMLEQLSQKEWSGYKTMTAYFVNYRVNAANQFEYDVVFHGVSTDDGETQAPIVQVNGPYTGMINEKIQFNSDGSKDTDGEIVSYLWDFGDGATSEAANPTHVYENEGTYKVTLTVKNNKGQESKGQTTATVQKGGQTGQEHAMIIPFNKPLKGSLIENDTNVYQFDITSPEEIDISVVNENQIGMTWVLYHESDKENYVAYGQEDGQTIKGKYNAKPGKYYLYVYKFDDEDGTYTVQVQNSTKTEIEPNNRPEEATMLPFHTPLSGSLMEDDHTDVYEFNVTSPKEIDISVLNENQIGMTWVLYHESDSQNYASFGQEDGNMINGKLNAKPGKYYLYVYKFENENGTYTVHVQ

SEQ ID NO: 7 - DNA, 2964 bp, Lysinibacillus fusiformis
  source 1..2964: mol_type = genomic DNA
gatacacagcaattgcaggagcagtactcgatggcagagcttaataatatgagcaatcgtgagcttatccatacgcttggcagtatccgttggtaccaaattacagacttattccaattcaatgatgacacaaaagctttttatcaaaatgaagagcgcatgcaagtaatcatcaatgaattagggaatagaggaaattcgtttacgaaggaagattcaaaggggatcgaaacatttgttgaggtattgcgttctgctttttatgtagcgttttataataatgaactaggctatttaaatgagagaagtttccaagataagtgtttaccagcattaaatgaaatagccaaaaatccaaactttaaacttggtacagatgagcaagataaagttgtatctgcctatggaaaattaataggtaatgcttctagtgatgtggaaaccgttcaacatgctacgaacattttaaaacaatataatgaaaatctttctacctatgaaagtgagaattcaaaaggacaagctatttacgatataatacacggcattgattatgatttgcagtcttatttatatgacactcgtaaagaggccaatacaacgatgtggtatgggaagattgatagcttcatagaggaagttaataacattgccctaatacataatgtgacggatagcaatagttggttaattaataatggcatttattatgcagggcgtttagggcagttccatagcaatcctaataagggtttagaagtcgttacacaagcgatgcatatgtatccctatttaagtgaagcttattttgtggcagtagagcaaattacgacaaattatggtggacgtgacttaaacggaaatacggttgatttacaaaaagtacgtgaagaaggaaaaaaacagtatctaccgaaaacatatacatttgatgatggatcaattgtattcaaaacgggagatcaagtaacggaagataaaattcaaagattatactgggctgcaaaagaggtaaaggcacaatatcatcgtgtaatcgggaatgatcaagcactagagcctggtaatgctgacgatatcttaaccgttgtcatttataactctcccgatcagtaccgattaaaccgacaattgtacggatatgaaacaaataatggtggtatttatattgaagagactggaacattctttacatatgaacgtacacctgagcaaagtatttatagcttagaagagctgttccgtcatgaatatacgcactttttacaaggtagatttgaggtgcctggtctattcgggacgggtgatatgtatcaaaatgagcgactaacatggttccaggaagggaatgcagaattttttgcagggtcaacacgtacaaatgacgttgtgcctcgtaagagcattattagtggattgtcacaggatccatcacaacgctatactgctgaacaaacaatgtttgccacatatggttcctgggatttttataattattcatttgcattacagtcttatatgtatacgcatcaattcgatatgtttgatagaattcaagatttaatccgcgcgaacgatgtgaaaaattatgatgcctatcgtgacactttaagtaaagattcacagctgaatatggaataccaagcatatatgcagcaattgatcgataaccaagaaacatacgaagtaccacaagtagcagaggattatttaatgccgcatgaaccaaaagcgttaaacgaagtacagcaagaaattgtcgatattgcacatgtgaaagatgcaaatatgacgaaacaccagtctcaattttttaatacgtttacactcgagggaacatatgtaggtagtgcaacacagggtgaatctcaagattggaaaacgatgagtaagcaagtaaaccaaatgctggagcaactgtctcaaaaagagtggagcggctataaaacaatgactgcgtactttgtcaactatcgtgtaaatgcggcaaaccagttcgagtatgatgtagtcttccatggcgtttccactgatgacggagaaacgcaagcaccaattgtacaagtaaatggtccatatactggcatgatcaatgaaaaaattcaatttaatagtgatgggtcaaaggatacggatggagaaatagtttcttatctttgggattttggtgatggcgcgacaagtgaagcagcaaatcctactcatgtatacgaaaatgaaggaacttacaaagtgacgttaaccgtgaaaaataataagggacaagaaagtaaagggcaaacaactgccactgtacagaaaggaggacagacagggcaagaacatgcgatgattattccatttaataaaccactaaaaggtagtttgatagaaaatgatacaaatgtctatcaatttgacattacatcgccagaagaaatagatatttctgtcgtaaatgaaaatcaaattggcatgacatgggtgctttatcatgaatctgataaggaaaactatgtagcgtatggacaggaagatggacagacaataaaaggtaagtacaatgcgaaaccaggaaagtattatttatacgtttataagtttgatgatgaagatggaacatataccgttcaagtacaaaatagtacaaaaacggagatagaaccaaacaatcgtccagaagaagccactatgcttccatttcatacaccactaagcggtagtttaatggaggatgatcatacggatgtatacgaattcaatgttacatctcctaaagaaatagatatatctgttttaaatgaaaaccaaattggcatgacatgggtgctttatcatgaatcagatagccaaaattatgcgtcttttggacaggaagacggaaacatgataaacggtaaattgaatgcaaagcctggaaagtattatttatatgtttataaatttgaaaatgagaacggaacatataccgttcatgtacagtaa

SEQ ID NO: 8 - DNA, 3219 bp, Lysinibacillus fusiformis
  source 1..3219: mol_type = genomic DNA
atgaagaaaaaatttacattcaatcagttgttaattggggttagtacaatggccatttcgttaggtggattacaggcggaagcatcggcagcagaaaaaacgccgtataatgtattacaaatgaaacccattggcatagaaatgtcgaaagatgaaatggtgcattcgacaatggctgaagaaacattatcctatgaagaacgtttagaaatgggagatttttcacaacgtccagcaccaattatggaacagatggatacacagcaattgcaggagcagtactcgatggcagagcttaataatatgagcaatcgtgagcttatccatacgcttggcagtatccgttggtaccaaattacagacttattccaattcaatgatgacacaaaagctttttatcaaaatgaagagcgcatgcaagtaatcatcaatgaattagggaatagaggaaattcgtttacgaaggaagattcaaaggggatcgaaacatttgttgaggtattgcgttctgctttttatgtagcgttttataataatgaactaggctatttaaatgagagaagtttccaagataagtgtttaccagcattaaatgaaatagccaaaaatccaaactttaaacttggtacagatgagcaagataaagttgtatctgcctatggaaaattaataggtaatgcttctagtgatgtggaaaccgttcaacatgctacgaacattttaaaacaatataatgaaaatctttctacctatgaaagtgagaattcaaaaggacaagctatttacgatataatacacggcattgattatgatttgcagtcttatttatatgacactcgtaaagaggccaatacaacgatgtggtatgggaagattgatagcttcatagaggaagttaataacattgccctaatacataatgtgacggatagcaatagttggttaattaataatggcatttattatgcagggcgtttagggcagttccatagcaatcctaataagggtttagaagtcgttacacaagcgatgcatatgtatccctatttaagtgaagcttattttgtggcagtagagcaaattacgacaaattatggtggacgtgacttaaacggaaatacggttgatttacaaaaagtacgtgaagaaggaaaaaaacagtatctaccgaaaacatatacatttgatgatggatcaattgtattcaaaacgggagatcaagtaacggaagataaaattcaaagattatactgggctgcaaaagaggtaaaggcacaatatcatcgtgtaatcgggaatgatcaagcactagagcctggtaatgctgacgatatcttaaccgttgtcatttataactctcccgatcagtaccgattaaaccgacaattgtacggatatgaaacaaataatggtggtatttatattgaagagactggaacattctttacatatgaacgtacacctgagcaaagtatttatagcttagaagagctgttccgtcatgaatatacgcactttttacaaggtagatttgaggtgcctggtctattcgggacgggtgatatgtatcaaaatgagcgactaacatggttccaggaagggaatgcagaattttttgcagggtcaacacgtacaaatgacgttgtgcctcgtaagagcattattagtggattgtcacaggatccatcacaacgctatactgctgaacaaacaatgtttgccacatatggttcctgggatttttataattattcatttgcattacagtcttatatgtatacgcatcaattcgatatgtttgatagaattcaagatttaatccgcgcgaacgatgtgaaaaattatgatgcctatcgtgacactttaagtaaagattcacagctgaatatggaataccaagcatatatgcagcaattgatcgataaccaagaaacatacgaagtaccacaagtagcagaggattatttaatgccgcatgaaccaaaagcgttaaacgaagtacagcaagaaattgtcgatattgcacatgtgaaagatgcaaatatgacgaaacaccagtctcaattttttaatacgtttacactcgagggaacatatgtaggtagtgcaacacagggtgaatctcaagattggaaaacgatgagtaagcaagtaaaccaaatgctggagcaactgtctcaaaaagagtggagcggctataaaacaatgactgcgtactttgtcaactatcgtgtaaatgcggcaaaccagttcgagtatgatgtagtcttccatggcgtttccactgatgacggagaaacgcaagcaccaattgtacaagtaaatggtccatatactggcatgatcaatgaaaaaattcaatttaatagtgatgggtcaaaggatacggatggagaaatagtttcttatctttgggattttggtgatggcgcgacaagtgaagcagcaaatcctactcatgtatacgaaaatgaaggaacttacaaagtgacgttaaccgtgaaaaataataagggacaagaaagtaaagggcaaacaactgccactgtacagaaaggaggacagacagggcaagaacatgcgatgattattccatttaataaaccactaaaaggtagtttgatagaaaatgatacaaatgtctatcaatttgacattacatcgccagaagaaatagatatttctgtcgtaaatgaaaatcaaattggcatgacatgggtgctttatcatgaatctgataaggaaaactatgtagcgtatggacaggaagatggacagacaataaaaggtaagtacaatgcgaaaccaggaaagtattatttatacgtttataagtttgatgatgaagatggaacatataccgttcaagtacaaaatagtacaaaaacggagatagaaccaaacaatcgtccagaagaagccactatgcttccatttcatacaccactaagcggtagtttaatggaggatgatcatacggatgtatacgaattcaatgttacatctcctaaagaaatagatatatctgttttaaatgaaaaccaaattggcatgacatgggtgctttatcatgaatcagatagccaaaattatgcgtcttttggacaggaagacggaaacatgataaacggtaaattgaatgcaaagcctggaaagtattatttatatgtttataaatttgaaaatgagaacggaacatataccgttcatgtacagtaa

SEQ ID NO: 9 - DNA, 21 bp, synthetic construct
  misc_feature 1..21: note = Forward primer
  source 1..21: mol_type = other DNA
ggaaacaatctaaatgtgtct

SEQ ID NO: 10 - DNA, 21 bp, synthetic construct
  misc_feature 1..21: note = Reverse primer
  source 1..21: mol_type = other DNA
ccgcctttaaaggctctccga